European Patent Specification EP 3 180 022 B1, published July 3, 2024. Title: AN IMPROVED EXPRESSION CASSETTE FOR PACKAGING AND EXPRESSION OF VARIANT FACTOR VIII FOR THE TREATMENT OF HEMOSTASIS DISORDERS. Applicant: THE CHILDREN'S HOSPITAL OF PHILADELPHIA SABATINO, Denise. Application PCT/US15/45142. The sequence listing filed with the application follows.

SEQUENCE LISTING (11 sequences)

SEQ ID NO: 1 - DNA, 4374 bp, Adeno-associated virus
atgcagattgagctgtcaacttgctttttcctgtgcctgctgagattttgtttttccgctactagaagatactacctgggggctgtggaactgtcttgggattacatgcagagtgacctgggagagctgccagtggacgcacgatttccacctagagtccctaaatcattccccttcaacaccagcgtggtctataagaaaacactgttcgtggagtttactgatcacctgttcaacatcgctaagcctcggccaccctggatgggactgctgggaccaacaatccaggcagaggtgtacgacaccgtggtcattacactgaaaaacatggcctcacaccccgtgagcctgcatgctgtgggcgtcagctactggaaggcttccgaaggggcagagtatgacgatcagacttcccagagagaaaaagaggacgataaggtgtttcctggcgggtctcatacctatgtgtggcaggtcctgaaagagaatggccccatggcttccgaccctctgtgcctgacctactcttatctgagtcacgtggacctggtcaaggatctgaacagcggactgatcggagcactgctggtgtgtagggaagggagcctggctaaggagaaaacccagacactgcataagttcattctgctgttcgccgtgtttgacgaaggaaaatcatggcacagcgagacaaagaatagtctgatgcaggaccgggatgccgcttcagccagagcttggcccaaaatgcacactgtgaacggctacgtcaatcgctcactgcctggactgatcggctgccaccgaaagagcgtgtattggcatgtcatcggaatgggcaccacacctgaagtgcactccattttcctggaggggcatacctttctggtccgcaaccaccgacaggcctccctggagatctctccaattaccttcctgacagctcagactctgctgatggatctgggacagttcctgctgttttgccacatcagctcccaccagcatgatggcatggaggcctacgtgaaagtggacagctgtcccgaggaacctcagctgaggatgaagaacaatgaggaagctgaagactatgacgatgacctgaccgactccgagatggatgtggtccgattcgatgacgataacagcccctcctttatccagattagatctgtggccaagaaacaccctaagacatgggtccattacatcgcagccgaggaagaggactgggattatgcaccactggtgctggcaccagacgatcgatcctacaaatctcagtatctgaacaatggaccacagcggattggcagaaagtacaagaaagtgaggttcatggcttataccgatgaaaccttcaagactcgcgaagcaatccagcacgagagcgggattctgggaccactgctgtacggagaagtgggggacaccctgctgatcatttttaagaaccaggccagcaggccttacaatatctatccacatggaattacagatgtgcgccctctgtacagccggagactgccaaagggcgtcaaacacctgaaggacttcccaatcctgcccggggaaatttttaagtataaatggactgtcaccgtcgaggatggccccactaagagcgaccctaggtgcctgacccgctactattctagtttcgtgaatatggaaagggatctggccagcggactgatcggcccactgctgatttgttacaaagagagcgtggatcagagaggcaaccagatcatgtccgacaagaggaatgtgattctgttcagtgtctttgacgaaaaccggtcatggtatctgaccgagaacatccagagattcctgcctaatccagccggagtgcagctggaagatcctgagtttcaggcttctaacatcatgcatagtattaatggctacgtgttcgacagtctgcagctgtcagtgtgtctgcacgaggtcgcttactggtatatcctgagcattggagcacagacagatttcctgagcgtgttcttttccggctacacttttaagcataaaatggtgtatgaggacacactgactctgttccccttcagcggcgaaaccgtgtttatgtccatggagaatcccgggctgtggatcctgggatgccacaacagcgatttcaggaatcgcgggatgactgccctgctgaaagtgtcaagctgtgacaagaacaccggagactactatgaagattcatacgaggacatcagcgcatatctgctgtccaaaaacaatgccattgaacccaggtcttttagtcagaatcctccagtgctgaagaggcaccagcgcgagatcacccgcactaccctgcagagtgatcaggaagagatcgactacgacgatacaatttctgtggaaatgaagaaagaggacttcgatatctatgacgaagatgagaaccagagtcctcgatcattccagaagaaaacccggcattactttattgctgcagtggagcgcctgtgggattatggcatgtcctctagtcctcacgtgctgcgaaatcgggcccagtcagggagcgtcccacagttcaagaaagtggtcttccaggagtttacagacggatcctttactcagccactgtaccggggcgaactgaacgagcacctggggctgctgggaccctatatcagagctgaagtggaggataacattatggtcaccttcagaaatcaggcatctaggccttacagtttttattcaagcctgatctcttacgaagaggaccagaggcagggagcagaaccacgaaaaaacttcgtgaagcctaatgagaccaaaacatacttttggaaggtgcagcaccatatggccccaacaaaagacgaattcgattgcaaggcatgggcctatttttctgacgtggatctggagaaggacgtccacagtggcctgatcgggccactgctggtgtgtcatactaacaccctgaatcccgcacacggcaggcaggtcactgtccaggaattcgccctgttctttaccatctttgatgagacaaaaagctggtacttcaccgaaaacatggagcgaaattgccgggctccatgtaatattcagatggaagaccccacattcaaggagaactaccgctttcatgccatcaatgggtatattatggatactctgcccggactggtcatggctcaggaccagagaatcaggtggtacctgctgagcatggggtccaacgagaatatccactcaattcatttcagcggacacgtgtttactgtccggaagaaagaagagtataaaatggccctgtacaacctgtatcccggcgtgttcgaaaccgtcgagatgctgcctagcaaggcagggatctggagagtggaatgcctgattggggagcacctgcatgccggaatgtctaccctgtttctggtgtacagtaataagtgtcagacacccctggggatggcttccggacatatccgggatttccagattaccgcatctggacagtacggccagtgggcccctaagctggctagactgcactattccgggtctatcaacgcttggtccacaaaagagcctttctcttggattaaggtggacctgctggcaccaatgatcattcatggcatcaaaactcagggggccaggcagaagttctcctctctgtacatctcacagtttatcatcatgtacagcctggatggcaagaaatggcagacataccgcggcaatagcacagggactctgatggtgttctttggcaacgtggacagttcagggatcaagcacaacattttcaatccccctatcattgctagatacatcaggctgcacccaacccattattctattcgaagtacactgcggatggaactgatggggtgcgatctgaacagttgttcaatgcccctgggaatggagtccaaggcaatctctgacgcccagattaccgctagctcctacttcactaatatgtttgctacctggagcccctccaaagcacgactgcatctgcagggacgaagcaacgcatggcgaccacaggtgaacaatcccaaggagtggctgcaggtcgattttcagaaaactatgaaggtgaccggagtcacaactcagggcgtgaaaagtctgctgacctcaatgtacgtcaaggagttcctgatctctagttcacaggacggccaccagtggacactgttctttcagaacggaaaggtgaaagtcttccagggcaatcaggattcctttacacctgtggtcaactctctggacccacccctgctgactcgctacctgcgaatccacccacagtcctgggtgcatcagattgcactgagaatggaagtcctgggctgcgaggcccaggacctgtattga

SEQ ID NO: 2 - DNA, 4374 bp, Adeno-associated virus
atgcagattgagctgtcaacttgctttttcctgtgcctgctgagattttgtttttccgctactagaagatactacctgggggctgtggaactgtcttgggattacatgcagagtgacctgggagagctgccagtggacgcacgatttccacctagagtccctaaatcattccccttcaacaccagcgtggtctataagaaaacactgttcgtggagtttactgatcacctgttcaacatcgctaagcctcggccaccctggatgggactgctgggaccaacaatccaggcagaggtgtacgacaccgtggtcattacactgaaaaacatggcctcacaccccgtgagcctgcatgctgtgggcgtcagctactggaaggcttccgaaggggcagagtatgacgatcagacttcccagagagaaaaagaggacgataaggtgtttcctggcgggtctcatacctatgtgtggcaggtcctgaaagagaatggccccatggcttccgaccctctgtgcctgacctactcttatctgagtcacgtggacctggtcaaggatctgaacagcggactgatcggagcactgctggtgtgtagggaagggagcctggctaaggagaaaacccagacactgcataagttcattctgctgttcgccgtgtttgacgaaggaaaatcatggcacagcgagacaaagaatagtctgatgcaggaccgggatgccgcttcagccagagcttggcccaaaatgcacactgtgaacggctacgtcaatcgctcactgcctggactgatcggctgccaccgaaagagcgtgtattggcatgtcatcggaatgggcaccacacctgaagtgcactccattttcctggaggggcatacctttctggtccgcaaccaccgacaggcctccctggagatctctccaattaccttcctgacagctcagactctgctgatggatctgggacagttcctgctgttttgccacatcagctcccaccagcatgatggcatggaggcctacgtgaaagtggacagctgtcccgaggaacctcagctgaggatgaagaacaatgaggaagctgaagactatgacgatgacctgaccgactccgagatggatgtggtccgattcgatgacgataacagcccctcctttatccagattagatctgtggccaagaaacaccctaagacatgggtccattacatcgcagccgaggaagaggactgggattatgcaccactggtgctggcaccagacgatcgatcctacaaatctcagtatctgaacaatggaccacagcggattggcagaaagtacaagaaagtgaggttcatggcttataccgatgaaaccttcaagactcgcgaagcaatccagcacgagagcgggattctgggaccactgctgtacggagaagtgggggacaccctgctgatcatttttaagaaccaggccagcaggccttacaatatctatccacatggaattacagatgtgcgccctctgtacagccggagactgccaaagggcgtcaaacacctgaaggacttcccaatcctgcccggggaaatttttaagtataaatggactgtcaccgtcgaggatggccccactaagagcgaccctaggtgcctgacccgctactattctagtttcgtgaatatggaaagggatctggccagcggactgatcggcccactgctgatttgttacaaagagagcgtggatcagagaggcaaccagatcatgtccgacaagaggaatgtgattctgttcagtgtctttgacgaaaaccggtcatggtatctgaccgagaacatccagagattcctgcctaatccagccggagtgcagctggaagatcctgagtttcaggcttctaacatcatgcatagtattaatggctacgtgttcgacagtctgcagctgtcagtgtgtctgcacgaggtcgcttactggtatatcctgagcattggagcacagacagatttcctgagcgtgttcttttccggctacacttttaagcataaaatggtgtatgaggacacactgactctgttccccttcagcggcgaaaccgtgtttatgtccatggagaatcccgggctgtggatcctgggatgccacaacagcgatttcaggaatcgcgggatgactgccctgctgaaagtgtcaagctgtgacaagaacaccggagactactatgaagattcatacgaggacatcagcgcatatctgctgtccaaaaacaatgccattgaacccaggtcttttagtcagaatcctccagtgctgaagcaccaccagcgcgagatcacccgcactaccctgcagagtgatcaggaagagatcgactacgacgatacaatttctgtggaaatgaagaaagaggacttcgatatctatgacgaagatgagaaccagagtcctcgatcattccagaagaaaacccggcattactttattgctgcagtggagcgcctgtgggattatggcatgtcctctagtcctcacgtgctgcgaaatcgggcccagtcagggagcgtcccacagttcaagaaagtggtcttccaggagtttacagacggatcctttactcagccactgtaccggggcgaactgaacgagcacctggggctgctgggaccctatatcagagctgaagtggaggataacattatggtcaccttcagaaatcaggcatctaggccttacagtttttattcaagcctgatctcttacgaagaggaccagaggcagggagcagaaccacgaaaaaacttcgtgaagcctaatgagaccaaaacatacttttggaaggtgcagcaccatatggccccaacaaaagacgaattcgattgcaaggcatgggcctatttttctgacgtggatctggagaaggacgtccacagtggcctgatcgggccactgctggtgtgtcatactaacaccctgaatcccgcacacggcaggcaggtcactgtccaggaattcgccctgttctttaccatctttgatgagacaaaaagctggtacttcaccgaaaacatggagcgaaattgccgggctccatgtaatattcagatggaagaccccacattcaaggagaactaccgctttcatgccatcaatgggtatattatggatactctgcccggactggtcatggctcaggaccagagaatcaggtggtacctgctgagcatggggtccaacgagaatatccactcaattcatttcagcggacacgtgtttactgtccggaagaaagaagagtataaaatggccctgtacaacctgtatcccggcgtgttcgaaaccgtcgagatgctgcctagcaaggcagggatctggagagtggaatgcctgattggggagcacctgcatgccggaatgtctaccctgtttctggtgtacagtaataagtgtcagacacccctggggatggcttccggacatatccgggatttccagattaccgcatctggacagtacggccagtgggcccctaagctggctagactgcactattccgggtctatcaacgcttggtccacaaaagagcctttctcttggattaaggtggacctgctggcaccaatgatcattcatggcatcaaaactcagggggccaggcagaagttctcctctctgtacatctcacagtttatcatcatgtacagcctggatggcaagaaatggcagacataccgcggcaatagcacagggactctgatggtgttctttggcaacgtggacagttcagggatcaagcacaacattttcaatccccctatcattgctagatacatcaggctgcacccaacccattattctattcgaagtacactgcggatggaactgatggggtgcgatctgaacagttgttcaatgcccctgggaatggagtccaaggcaatctctgacgcccagattaccgctagctcctacttcactaatatgtttgctacctggagcccctccaaagcacgactgcatctgcagggacgaagcaacgcatggcgaccacaggtgaacaatcccaaggagtggctgcaggtcgattttcagaaaactatgaaggtgaccggagtcacaactcagggcgtgaaaagtctgctgacctcaatgtacgtcaaggagttcctgatctctagttcacaggacggccaccagtggacactgttctttcagaacggaaaggtgaaagtcttccagggcaatcaggattcctttacacctgtggtcaactctctggacccacccctgctgactcgctacctgcgaatccacccacagtcctgggtgcatcagattgcactgagaatggaagtcctgggctgcgaggcccaggacctgtattga

SEQ ID NO: 3 - DNA, 4362 bp, Adeno-associated virus
atgcagattgagctgtcaacttgctttttcctgtgcctgctgagattttgtttttccgctactagaagatactacctgggggctgtggaactgtcttgggattacatgcagagtgacctgggagagctgccagtggacgcacgatttccacctagagtccctaaatcattccccttcaacaccagcgtggtctataagaaaacactgttcgtggagtttactgatcacctgttcaacatcgctaagcctcggccaccctggatgggactgctgggaccaacaatccaggcagaggtgtacgacaccgtggtcattacactgaaaaacatggcctcacaccccgtgagcctgcatgctgtgggcgtcagctactggaaggcttccgaaggggcagagtatgacgatcagacttcccagagagaaaaagaggacgataaggtgtttcctggcgggtctcatacctatgtgtggcaggtcctgaaagagaatggccccatggcttccgaccctctgtgcctgacctactcttatctgagtcacgtggacctggtcaaggatctgaacagcggactgatcggagcactgctggtgtgtagggaagggagcctggctaaggagaaaacccagacactgcataagttcattctgctgttcgccgtgtttgacgaaggaaaatcatggcacagcgagacaaagaatagtctgatgcaggaccgggatgccgcttcagccagagcttggcccaaaatgcacactgtgaacggctacgtcaatcgctcactgcctggactgatcggctgccaccgaaagagcgtgtattggcatgtcatcggaatgggcaccacacctgaagtgcactccattttcctggaggggcatacctttctggtccgcaaccaccgacaggcctccctggagatctctccaattaccttcctgacagctcagactctgctgatggatctgggacagttcctgctgttttgccacatcagctcccaccagcatgatggcatggaggcctacgtgaaagtggacagctgtcccgaggaacctcagctgaggatgaagaacaatgaggaagctgaagactatgacgatgacctgaccgactccgagatggatgtggtccgattcgatgacgataacagcccctcctttatccagattagatctgtggccaagaaacaccctaagacatgggtccattacatcgcagccgaggaagaggactgggattatgcaccactggtgctggcaccagacgatcgatcctacaaatctcagtatctgaacaatggaccacagcggattggcagaaagtacaagaaagtgaggttcatggcttataccgatgaaaccttcaagactcgcgaagcaatccagcacgagagcgggattctgggaccactgctgtacggagaagtgggggacaccctgctgatcatttttaagaaccaggccagcaggccttacaatatctatccacatggaattacagatgtgcgccctctgtacagccggagactgccaaagggcgtcaaacacctgaaggacttcccaatcctgcccggggaaatttttaagtataaatggactgtcaccgtcgaggatggccccactaagagcgaccctaggtgcctgacccgctactattctagtttcgtgaatatggaaagggatctggccagcggactgatcggcccactgctgatttgttacaaagagagcgtggatcagagaggcaaccagatcatgtccgacaagaggaatgtgattctgttcagtgtctttgacgaaaaccggtcatggtatctgaccgagaacatccagagattcctgcctaatccagccggagtgcagctggaagatcctgagtttcaggcttctaacatcatgcatagtattaatggctacgtgttcgacagtctgcagctgtcagtgtgtctgcacgaggtcgcttactggtatatcctgagcattggagcacagacagatttcctgagcgtgttcttttccggctacacttttaagcataaaatggtgtatgaggacacactgactctgttccccttcagcggcgaaaccgtgtttatgtccatggagaatcccgggctgtggatcctgggatgccacaacagcgatttcaggaatcgcgggatgactgccctgctgaaagtgtcaagctgtgacaagaacaccggagactactatgaagattcatacgaggacatcagcgcatatctgctgtccaaaaacaatgccattgaacccaggtcttttagtcagaatcctccagtgctgaaggagatcacccgcactaccctgcagagtgatcaggaagagatcgactacgacgatacaatttctgtggaaatgaagaaagaggacttcgatatctatgacgaagatgagaaccagagtcctcgatcattccagaagaaaacccggcattactttattgctgcagtggagcgcctgtgggattatggcatgtcctctagtcctcacgtgctgcgaaatcgggcccagtcagggagcgtcccacagttcaagaaagtggtcttccaggagtttacagacggatcctttactcagccactgtaccggggcgaactgaacgagcacctggggctgctgggaccctatatcagagctgaagtggaggataacattatggtcaccttcagaaatcaggcatctaggccttacagtttttattcaagcctgatctcttacgaagaggaccagaggcagggagcagaaccacgaaaaaacttcgtgaagcctaatgagaccaaaacatacttttggaaggtgcagcaccatatggccccaacaaaagacgaattcgattgcaaggcatgggcctatttttctgacgtggatctggagaaggacgtccacagtggcctgatcgggccactgctggtgtgtcatactaacaccctgaatcccgcacacggcaggcaggtcactgtccaggaattcgccctgttctttaccatctttgatgagacaaaaagctggtacttcaccgaaaacatggagcgaaattgccgggctccatgtaatattcagatggaagaccccacattcaaggagaactaccgctttcatgccatcaatgggtatattatggatactctgcccggactggtcatggctcaggaccagagaatcaggtggtacctgctgagcatggggtccaacgagaatatccactcaattcatttcagcggacacgtgtttactgtccggaagaaagaagagtataaaatggccctgtacaacctgtatcccggcgtgttcgaaaccgtcgagatgctgcctagcaaggcagggatctggagagtggaatgcctgattggggagcacctgcatgccggaatgtctaccctgtttctggtgtacagtaataagtgtcagacacccctggggatggcttccggacatatccgggatttccagattaccgcatctggacagtacggccagtgggcccctaagctggctagactgcactattccgggtctatcaacgcttggtccacaaaagagcctttctcttggattaaggtggacctgctggcaccaatgatcattcatggcatcaaaactcagggggccaggcagaagttctcctctctgtacatctcacagtttatcatcatgtacagcctggatggcaagaaatggcagacataccgcggcaatagcacagggactctgatggtgttctttggcaacgtggacagttcagggatcaagcacaacattttcaatccccctatcattgctagatacatcaggctgcacccaacccattattctattcgaagtacactgcggatggaactgatggggtgcgatctgaacagttgttcaatgcccctgggaatggagtccaaggcaatctctgacgcccagattaccgctagctcctacttcactaatatgtttgctacctggagcccctccaaagcacgactgcatctgcagggacgaagcaacgcatggcgaccacaggtgaacaatcccaaggagtggctgcaggtcgattttcagaaaactatgaaggtgaccggagtcacaactcagggcgtgaaaagtctgctgacctcaatgtacgtcaaggagttcctgatctctagttcacaggacggccaccagtggacactgttctttcagaacggaaaggtgaaagtcttccagggcaatcaggattcctttacacctgtggtcaactctctggacccacccctgctgactcgctacctgcgaatccacccacagtcctgggtgcatcagattgcactgagaatggaagtcctgggctgcgaggcccaggacctgtattga

SEQ ID NO: 4 - DNA, 4371 bp, Adeno-associated virus
atgcagattgagctgtcaacttgctttttcctgtgcctgctgagattttgtttttccgctactagaagatactacctgggggctgtggaactgtcttgggattacatgcagagtgacctgggagagctgccagtggacgcacgatttccacctagagtccctaaatcattccccttcaacaccagcgtggtctataagaaaacactgttcgtggagtttactgatcacctgttcaacatcgctaagcctcggccaccctggatgggactgctgggaccaacaatccaggcagaggtgtacgacaccgtggtcattacactgaaaaacatggcctcacaccccgtgagcctgcatgctgtgggcgtcagctactggaaggcttccgaaggggcagagtatgacgatcagacttcccagagagaaaaagaggacgataaggtgtttcctggcgggtctcatacctatgtgtggcaggtcctgaaagagaatggccccatggcttccgaccctctgtgcctgacctactcttatctgagtcacgtggacctggtcaaggatctgaacagcggactgatcggagcactgctggtgtgtagggaagggagcctggctaaggagaaaacccagacactgcataagttcattctgctgttcgccgtgtttgacgaaggaaaatcatggcacagcgagacaaagaatagtctgatgcaggaccgggatgccgcttcagccagagcttggcccaaaatgcacactgtgaacggctacgtcaatcgctcactgcctggactgatcggctgccaccgaaagagcgtgtattggcatgtcatcggaatgggcaccacacctgaagtgcactccattttcctggaggggcatacctttctggtccgcaaccaccgacaggcctccctggagatctctccaattaccttcctgacagctcagactctgctgatggatctgggacagttcctgctgttttgccacatcagctcccaccagcatgatggcatggaggcctacgtgaaagtggacagctgtcccgaggaacctcagctgaggatgaagaacaatgaggaagctgaagactatgacgatgacctgaccgactccgagatggatgtggtccgattcgatgacgataacagcccctcctttatccagattagatctgtggccaagaaacaccctaagacatgggtccattacatcgcagccgaggaagaggactgggattatgcaccactggtgctggcaccagacgatcgatcctacaaatctcagtatctgaacaatggaccacagcggattggcagaaagtacaagaaagtgaggttcatggcttataccgatgaaaccttcaagactcgcgaagcaatccagcacgagagcgggattctgggaccactgctgtacggagaagtgggggacaccctgctgatcatttttaagaaccaggccagcaggccttacaatatctatccacatggaattacagatgtgcgccctctgtacagccggagactgccaaagggcgtcaaacacctgaaggacttcccaatcctgcccggggaaatttttaagtataaatggactgtcaccgtcgaggatggccccactaagagcgaccctaggtgcctgacccgctactattctagtttcgtgaatatggaaagggatctggccagcggactgatcggcccactgctgatttgttacaaagagagcgtggatcagagaggcaaccagatcatgtccgacaagaggaatgtgattctgttcagtgtctttgacgaaaaccggtcatggtatctgaccgagaacatccagagattcctgcctaatccagccggagtgcagctggaagatcctgagtttcaggcttctaacatcatgcatagtattaatggctacgtgttcgacagtctgcagctgtcagtgtgtctgcacgaggtcgcttactggtatatcctgagcattggagcacagacagatttcctgagcgtgttcttttccggctacacttttaagcataaaatggtgtatgaggacacactgactctgttccccttcagcggcgaaaccgtgtttatgtccatggagaatcccgggctgtggatcctgggatgccacaacagcgatttcaggaatcgcgggatgactgccctgctgaaagtgtcaagctgtgacaagaacaccggagactactatgaagattcatacgaggacatcagcgcatatctgctgtccaaaaacaatgccattgaacccaggtcttttagtcagaatcctccagtgctgaagcaccagcgcgagatcacccgcactaccctgcagagtgatcaggaagagatcgactacgacgatacaatttctgtggaaatgaagaaagaggacttcgatatctatgacgaagatgagaaccagagtcctcgatcattccagaagaaaacccggcattactttattgctgcagtggagcgcctgtgggattatggcatgtcctctagtcctcacgtgctgcgaaatcgggcccagtcagggagcgtcccacagttcaagaaagtggtcttccaggagtttacagacggatcctttactcagccactgtaccggggcgaactgaacgagcacctggggctgctgggaccctatatcagagctgaagtggaggataacattatggtcaccttcagaaatcaggcatctaggccttacagtttttattcaagcctgatctcttacgaagaggaccagaggcagggagcagaaccacgaaaaaacttcgtgaagcctaatgagaccaaaacatacttttggaaggtgcagcaccatatggccccaacaaaagacgaattcgattgcaaggcatgggcctatttttctgacgtggatctggagaaggacgtccacagtggcctgatcgggccactgctggtgtgtcatactaacaccctgaatcccgcacacggcaggcaggtcactgtccaggaattcgccctgttctttaccatctttgatgagacaaaaagctggtacttcaccgaaaacatggagcgaaattgccgggctccatgtaatattcagatggaagaccccacattcaaggagaactaccgctttcatgccatcaatgggtatattatggatactctgcccggactggtcatggctcaggaccagagaatcaggtggtacctgctgagcatggggtccaacgagaatatccactcaattcatttcagcggacacgtgtttactgtccggaagaaagaagagtataaaatggccctgtacaacctgtatcccggcgtgttcgaaaccgtcgagatgctgcctagcaaggcagggatctggagagtggaatgcctgattggggagcacctgcatgccggaatgtctaccctgtttctggtgtacagtaataagtgtcagacacccctggggatggcttccggacatatccgggatttccagattaccgcatctggacagtacggccagtgggcccctaagctggctagactgcactattccgggtctatcaacgcttggtccacaaaagagcctttctcttggattaaggtggacctgctggcaccaatgatcattcatggcatcaaaactcagggggccaggcagaagttctcctctctgtacatctcacagtttatcatcatgtacagcctggatggcaagaaatggcagacataccgcggcaatagcacagggactctgatggtgttctttggcaacgtggacagttcagggatcaagcacaacattttcaatccccctatcattgctagatacatcaggctgcacccaacccattattctattcgaagtacactgcggatggaactgatggggtgcgatctgaacagttgttcaatgcccctgggaatggagtccaaggcaatctctgacgcccagattaccgctagctcctacttcactaatatgtttgctacctggagcccctccaaagcacgactgcatctgcagggacgaagcaacgcatggcgaccacaggtgaacaatcccaaggagtggctgcaggtcgattttcagaaaactatgaaggtgaccggagtcacaactcagggcgtgaaaagtctgctgacctcaatgtacgtcaaggagttcctgatctctagttcacaggacggccaccagtggacactgttctttcagaacggaaaggtgaaagtcttccagggcaatcaggattcctttacacctgtggtcaactctctggacccacccctgctgactcgctacctgcgaatccacccacagtcctgggtgcatcagattgcactgagaatggaagtcctgggctgcgaggcccaggacctgtattga

SEQ ID NO: 5 - DNA, 4368 bp, Adeno-associated virus
atgcagattgagctgtcaacttgctttttcctgtgcctgctgagattttgtttttccgctactagaagatactacctgggggctgtggaactgtcttgggattacatgcagagtgacctgggagagctgccagtggacgcacgatttccacctagagtccctaaatcattccccttcaacaccagcgtggtctataagaaaacactgttcgtggagtttactgatcacctgttcaacatcgctaagcctcggccaccctggatgggactgctgggaccaacaatccaggcagaggtgtacgacaccgtggtcattacactgaaaaacatggcctcacaccccgtgagcctgcatgctgtgggcgtcagctactggaaggcttccgaaggggcagagtatgacgatcagacttcccagagagaaaaagaggacgataaggtgtttcctggcgggtctcatacctatgtgtggcaggtcctgaaagagaatggccccatggcttccgaccctctgtgcctgacctactcttatctgagtcacgtggacctggtcaaggatctgaacagcggactgatcggagcactgctggtgtgtagggaagggagcctggctaaggagaaaacccagacactgcataagttcattctgctgttcgccgtgtttgacgaaggaaaatcatggcacagcgagacaaagaatagtctgatgcaggaccgggatgccgcttcagccagagcttggcccaaaatgcacactgtgaacggctacgtcaatcgctcactgcctggactgatcggctgccaccgaaagagcgtgtattggcatgtcatcggaatgggcaccacacctgaagtgcactccattttcctggaggggcatacctttctggtccgcaaccaccgacaggcctccctggagatctctccaattaccttcctgacagctcagactctgctgatggatctgggacagttcctgctgttttgccacatcagctcccaccagcatgatggcatggaggcctacgtgaaagtggacagctgtcccgaggaacctcagctgaggatgaagaacaatgaggaagctgaagactatgacgatgacctgaccgactccgagatggatgtggtccgattcgatgacgataacagcccctcctttatccagattagatctgtggccaagaaacaccctaagacatgggtccattacatcgcagccgaggaagaggactgggattatgcaccactggtgctggcaccagacgatcgatcctacaaatctcagtatctgaacaatggaccacagcggattggcagaaagtacaagaaagtgaggttcatggcttataccgatgaaaccttcaagactcgcgaagcaatccagcacgagagcgggattctgggaccactgctgtacggagaagtgggggacaccctgctgatcatttttaagaaccaggccagcaggccttacaatatctatccacatggaattacagatgtgcgccctctgtacagccggagactgccaaagggcgtcaaacacctgaaggacttcccaatcctgcccggggaaatttttaagtataaatggactgtcaccgtcgaggatggccccactaagagcgaccctaggtgcctgacccgctactattctagtttcgtgaatatggaaagggatctggccagcggactgatcggcccactgctgatttgttacaaagagagcgtggatcagagaggcaaccagatcatgtccgacaagaggaatgtgattctgttcagtgtctttgacgaaaaccggtcatggtatctgaccgagaacatccagagattcctgcctaatccagccggagtgcagctggaagatcctgagtttcaggcttctaacatcatgcatagtattaatggctacgtgttcgacagtctgcagctgtcagtgtgtctgcacgaggtcgcttactggtatatcctgagcattggagcacagacagatttcctgagcgtgttcttttccggctacacttttaagcataaaatggtgtatgaggacacactgactctgttccccttcagcggcgaaaccgtgtttatgtccatggagaatcccgggctgtggatcctgggatgccacaacagcgatttcaggaatcgcgggatgactgccctgctgaaagtgtcaagctgtgacaagaacaccggagactactatgaagattcatacgaggacatcagcgcatatctgctgtccaaaaacaatgccattgaacccaggtcttttagtcagaatcctccagtgctgaagcagcgcgagatcacccgcactaccctgcagagtgatcaggaagagatcgactacgacgatacaatttctgtggaaatgaagaaagaggacttcgatatctatgacgaagatgagaaccagagtcctcgatcattccagaagaaaacccggcattactttattgctgcagtggagcgcctgtgggattatggcatgtcctctagtcctcacgtgctgcgaaatcgggcccagtcagggagcgtcccacagttcaagaaagtggtcttccaggagtttacagacggatcctttactcagccactgtaccggggcgaactgaacgagcacctggggctgctgggaccctatatcagagctgaagtggaggataacattatggtcaccttcagaaatcaggcatctaggccttacagtttttattcaagcctgatctcttacgaagaggaccagaggcagggagcagaaccacgaaaaaacttcgtgaagcctaatgagaccaaaacatacttttggaaggtgcagcaccatatggccccaacaaaagacgaattcgattgcaaggcatgggcctatttttctgacgtggatctggagaaggacgtccacagtggcctgatcgggccactgctggtgtgtcatactaacaccctgaatcccgcacacggcaggcaggtcactgtccaggaattcgccctgttctttaccatctttgatgagacaaaaagctggtacttcaccgaaaacatggagcgaaattgccgggctccatgtaatattcagatggaagaccccacattcaaggagaactaccgctttcatgccatcaatgggtatattatggatactctgcccggactggtcatggctcaggaccagagaatcaggtggtacctgctgagcatggggtccaacgagaatatccactcaattcatttcagcggacacgtgtttactgtccggaagaaagaagagtataaaatggccctgtacaacctgtatcccggcgtgttcgaaaccgtcgagatgctgcctagcaaggcagggatctggagagtggaatgcctgattggggagcacctgcatgccggaatgtctaccctgtttctggtgtacagtaataagtgtcagacacccctggggatggcttccggacatatccgggatttccagattaccgcatctggacagtacggccagtgggcccctaagctggctagactgcactattccgggtctatcaacgcttggtccacaaaagagcctttctcttggattaaggtggacctgctggcaccaatgatcattcatggcatcaaaactcagggggccaggcagaagttctcctctctgtacatctcacagtttatcatcatgtacagcctggatggcaagaaatggcagacataccgcggcaatagcacagggactctgatggtgttctttggcaacgtggacagttcagggatcaagcacaacattttcaatccccctatcattgctagatacatcaggctgcacccaacccattattctattcgaagtacactgcggatggaactgatggggtgcgatctgaacagttgttcaatgcccctgggaatggagtccaaggcaatctctgacgcccagattaccgctagctcctacttcactaatatgtttgctacctggagcccctccaaagcacgactgcatctgcagggacgaagcaacgcatggcgaccacaggtgaacaatcccaaggagtggctgcaggtcgattttcagaaaactatgaaggtgaccggagtcacaactcagggcgtgaaaagtctgctgacctcaatgtacgtcaaggagttcctgatctctagttcacaggacggccaccagtggacactgttctttcagaacggaaaggtgaaagtcttccagggcaatcaggattcctttacacctgtggtcaactctctggacccacccctgctgactcgctacctgcgaatccacccacagtcctgggtgcatcagattgcactgagaatggaagtcctgggctgcgaggcccaggacctgtattga

SEQ ID NO: 6 - DNA, 4365 bp, Adeno-associated virus
atgcagattgagctgtcaacttgctttttcctgtgcctgctgagattttgtttttccgctactagaagatactacctgggggctgtggaactgtcttgggattacatgcagagtgacctgggagagctgccagtggacgcacgatttccacctagagtccctaaatcattccccttcaacaccagcgtggtctataagaaaacactgttcgtggagtttactgatcacctgttcaacatcgctaagcctcggccaccctggatgggactgctgggaccaacaatccaggcagaggtgtacgacaccgtggtcattacactgaaaaacatggcctcacaccccgtgagcctgcatgctgtgggcgtcagctactggaaggcttccgaaggggcagagtatgacgatcagacttcccagagagaaaaagaggacgataaggtgtttcctggcgggtctcatacctatgtgtggcaggtcctgaaagagaatggccccatggcttccgaccctctgtgcctgacctactcttatctgagtcacgtggacctggtcaaggatctgaacagcggactgatcggagcactgctggtgtgtagggaagggagcctggctaaggagaaaacccagacactgcataagttcattctgctgttcgccgtgtttgacgaaggaaaatcatggcacagcgagacaaagaatagtctgatgcaggaccgggatgccgcttcagccagagcttggcccaaaatgcacactgtgaacggctacgtcaatcgctcactgcctggactgatcggctgccaccgaaagagcgtgtattggcatgtcatcggaatgggcaccacacctgaagtgcactccattttcctggaggggcatacctttctggtccgcaaccaccgacaggcctccctggagatctctccaattaccttcctgacagctcagactctgctgatggatctgggacagttcctgctgttttgccacatcagctcccaccagcatgatggcatggaggcctacgtgaaagtggacagctgtcccgaggaacctcagctgaggatgaagaacaatgaggaagctgaagactatgacgatgacctgaccgactccgagatggatgtggtccgattcgatgacgataacagcccctcctttatccagattagatctgtggccaagaaacaccctaagacatgggtccattacatcgcagccgaggaagaggactgggattatgcaccactggtgctggcaccagacgatcgatcctacaaatctcagtatctgaacaatggaccacagcggattggcagaaagtacaagaaagtgaggttcatggcttataccgatgaaaccttcaagactcgcgaagcaatccagcacgagagcgggattctgggaccactgctgtacggagaagtgggggacaccctgctgatcatttttaagaaccaggccagcaggccttacaatatctatccacatggaattacagatgtgcgccctctgtacagccggagactgccaaagggcgtcaaacacctgaaggacttcccaatcctgcccggggaaatttttaagtataaatggactgtcaccgtcgaggatggccccactaagagcgaccctaggtgcctgacccgctactattctagtttcgtgaatatggaaagggatctggccagcggactgatcggcccactgctgatttgttacaaagagagcgtggatcagagaggcaaccagatcatgtccgacaagaggaatgtgattctgttcagtgtctttgacgaaaaccggtcatggtatctgaccgagaacatccagagattcctgcctaatccagccggagtgcagctggaagatcctgagtttcaggcttctaacatcatgcatagtattaatggctacgtgttcgacagtctgcagctgtcagtgtgtctgcacgaggtcgcttactggtatatcctgagcattggagcacagacagatttcctgagcgtgttcttttccggctacacttttaagcataaaatggtgtatgaggacacactgactctgttccccttcagcggcgaaaccgtgtttatgtccatggagaatcccgggctgtggatcctgggatgccacaacagcgatttcaggaatcgcgggatgactgccctgctgaaagtgtcaagctgtgacaagaacaccggagactactatgaagattcatacgaggacatcagcgcatatctgctgtccaaaaacaatgccattgaacccaggtcttttagtcagaatcctccagtgctgaagcgcgagatcacccgcactaccctgcagagtgatcaggaagagatcgactacgacgatacaatttctgtggaaatgaagaaagaggacttcgatatctatgacgaagatgagaaccagagtcctcgatcattccagaagaaaacccggcattactttattgctgcagtggagcgcctgtgggattatggcatgtcctctagtcctcacgtgctgcgaaatcgggcccagtcagggagcgtcccacagttcaagaaagtggtcttccaggagtttacagacggatcctttactcagccactgtaccggggcgaactgaacgagcacctggggctgctgggaccctatatcagagctgaagtggaggataacattatggtcaccttcagaaatcaggcatctaggccttacagtttttattcaagcctgatctcttacgaagaggaccagaggcagggagcagaaccacgaaaaaacttcgtgaagcctaatgagaccaaaacatacttttggaaggtgcagcaccatatggccccaacaaaagacgaattcgattgcaaggcatgggcctatttttctgacgtggatctggagaaggacgtccacagtggcctgatcgggccactgctggtgtgtcatactaacaccctgaatcccgcacacggcaggcaggtcactgtccaggaattcgccctgttctttaccatctttgatgagacaaaaagctggtacttcaccgaaaacatggagcgaaattgccgggctccatgtaatattcagatggaagaccccacattcaaggagaactaccgctttcatgccatcaatgggtatattatggatactctgcccggactggtcatggctcaggaccagagaatcaggtggtacctgctgagcatggggtccaacgagaatatccactcaattcatttcagcggacacgtgtttactgtccggaagaaagaagagtataaaatggccctgtacaacctgtatcccggcgtgttcgaaaccgtcgagatgctgcctagcaaggcagggatctggagagtggaatgcctgattggggagcacctgcatgccggaatgtctaccctgtttctggtgtacagtaataagtgtcagacacccctggggatggcttccggacatatccgggatttccagattaccgcatctggacagtacggccagtgggcccctaagctggctagactgcactattccgggtctatcaacgcttggtccacaaaagagcctttctcttggattaaggtggacctgctggcaccaatgatcattcatggcatcaaaactcagggggccaggcagaagttctcctctctgtacatctcacagtttatcatcatgtacagcctggatggcaagaaatggcagacataccgcggcaatagcacagggactctgatggtgttctttggcaacgtggacagttcagggatcaagcacaacattttcaatccccctatcattgctagatacatcaggctgcacccaacccattattctattcgaagtacactgcggatggaactgatggggtgcgatctgaacagttgttcaatgcccctgggaatggagtccaaggcaatctctgacgcccagattaccgctagctcctacttcactaatatgtttgctacctggagcccctccaaagcacgactgcatctgcagggacgaagcaacgcatggcgaccacaggtgaacaatcccaaggagtggctgcaggtcgattttcagaaaactatgaaggtgaccggagtcacaactcagggcgtgaaaagtctgctgacctcaatgtacgtcaaggagttcctgatctctagttcacaggacggccaccagtggacactgttctttcagaacggaaaggtgaaagtcttccagggcaatcaggattcctttacacctgtggtcaactctctggacccacccctgctgactcgctacctgcgaatccacccacagtcctgggtgcatcagattgcactgagaatggaagtcctgggctgcgaggcccaggacctgtattga

SEQ ID NO: 7 - DNA, 4371 bp, Adeno-associated virus
atgcagattgagctgtcaacttgctttttcctgtgcctgctgagattttgtttttccgctactagaagatactacctgggggctgtggaactgtcttgggattacatgcagagtgacctgggagagctgccagtggacgcacgatttccacctagagtccctaaatcattccccttcaacaccagcgtggtctataagaaaacactgttcgtggagtttactgatcacctgttcaacatcgctaagcctcggccaccctggatgggactgctgggaccaacaatccaggcagaggtgtacgacaccgtggtcattacactgaaaaacatggcctcacaccccgtgagcctgcatgctgtgggcgtcagctactggaaggcttccgaaggggcagagtatgacgatcagacttcccagagagaaaaagaggacgataaggtgtttcctggcgggtctcatacctatgtgtggcaggtcctgaaagagaatggccccatggcttccgaccctctgtgcctgacctactcttatctgagtcacgtggacctggtcaaggatctgaacagcggactgatcggagcactgctggtgtgtagggaagggagcctggctaaggagaaaacccagacactgcataagttcattctgctgttcgccgtgtttgacgaaggaaaatcatggcacagcgagacaaagaatagtctgatgcaggaccgggatgccgcttcagccagagcttggcccaaaatgcacactgtgaacggctacgtcaatcgctcactgcctggactgatcggctgccaccgaaagagcgtgtattggcatgtcatcggaatgggcaccacacctgaagtgcactccattttcctggaggggcatacctttctggtccgcaaccaccgacaggcctccctggagatctctccaattaccttcctgacagctcagactctgctgatggatctgggacagttcctgctgttttgccacatcagctcccaccagcatgatggcatggaggcctacgtgaaagtggacagctgtcccgaggaacctcagctgaggatgaagaacaatgaggaagctgaagactatgacgatgacctgaccgactccgagatggatgtggtccgattcgatgacgataacagcccctcctttatccagattagatctgtggccaagaaacaccctaagacatgggtccattacatcgcagccgaggaagaggactgggattatgcaccactggtgctggcaccagacgatcgatcctacaaatctcagtatctgaacaatggaccacagcggattggcagaaagtacaagaaagtgaggttcatggcttataccgatgaaaccttcaagactcgcgaagcaatccagcacgagagcgggattctgggaccactgctgtacggagaagtgggggacaccctgctgatcatttttaagaaccaggccagcaggccttacaatatctatccacatggaattacagatgtgcgccctctgtacagccggagactgccaaagggcgtcaaacacctgaaggacttcccaatcctgcccggggaaatttttaagtataaatggactgtcaccgtcgaggatggccccactaagagcgaccctaggtgcctgacccgctactattctagtttcgtgaatatggaaagggatctggccagcggactgatcggcccactgctgatttgttacaaagagagcgtggatcagagaggcaaccagatcatgtccgacaagaggaatgtgattctgttcagtgtctttgacgaaaaccggtcatggtatctgaccgagaacatccagagattcctgcctaatccagccggagtgcagctggaagatcctgagtttcaggcttctaacatcatgcatagtattaatggctacgtgttcgacagtctgcagctgtcagtgtgtctgcacgaggtcgcttactggtatatcctgagcattggagcacagacagatttcctgagcgtgttcttttccggctacacttttaagcataaaatggtgtatgaggacacactgactctgttccccttcagcggcgaaaccgtgtttatgtccatggagaatcccgggctgtggatcctgggatgccacaacagcgatttcaggaatcgcgggatgactgccctgctgaaagtgtcaagctgtgacaagaacaccggagactactatgaagattcatacgaggacatcagcgcatatctgctgtccaaaaacaatgccattgaacccaggtcttttagtcagaatcctccagtgctgaagaggcaccaggagatcacccgcactaccctgcagagtgatcaggaagagatcgactacgacgatacaatttctgtggaaatgaagaaagaggacttcgatatctatgacgaagatgagaaccagagtcctcgatcattccagaagaaaacccggcattactttattgctgcagtggagcgcctgtgggattatggcatgtcctctagtcctcacgtgctgcgaaatcgggcccagtcagggagcgtcccacagttcaagaaagtggtcttccaggagtttacagacggatcctttactcagccactgtaccggggcgaactgaacgagcacctggggctgctgggaccctatatcagagctgaagtggaggataacattatggtcaccttcagaaatcaggcatctaggccttacagtttttattcaagcctgatctcttacgaagaggaccagaggcagggagcagaaccacgaaaaaacttcgtgaagcctaatgagaccaaaacatacttttggaaggtgcagcaccatatggccccaacaaaagacgaattcgattgcaaggcatgggcctatttttctgacgtggatctggagaaggacgtccacagtggcctgatcgggccactgctggtgtgtcatactaacaccctgaatcccgcacacggcaggcaggtcactgtccaggaattcgccctgttctttaccatctttgatgagacaaaaagctggtacttcaccgaaaacatggagcgaaattgccgggctccatgtaatattcagatggaagaccccacattcaaggagaactaccgctttcatgccatcaatgggtatattatggatactctgcccggactggtcatggctcaggaccagagaatcaggtggtacctgctgagcatggggtccaacgagaatatccactcaattcatttcagcggacacgtgtttactgtccggaagaaagaagagtataaaatggccctgtacaacctgtatcccggcgtgttcgaaaccgtcgagatgctgcctagcaaggcagggatctggagagtggaatgcctgattggggagcacctgcatgccggaatgtctaccctgtttctggtgtacagtaataagtgtcagacacccctggggatggcttccggacatatccgggatttccagattaccgcatctggacagtacggccagtgggcccctaagctggctagactgcactattccgggtctatcaacgcttggtccacaaaagagcctttctcttggattaaggtggacctgctggcaccaatgatcattcatggcatcaaaactcagggggccaggcagaagttctcctctctgtacatctcacagtttatcatcatgtacagcctggatggcaagaaatggcagacataccgcggcaatagcacagggactctgatggtgttctttggcaacgtggacagttcagggatcaagcacaacattttcaatccccctatcattgctagatacatcaggctgcacccaacccattattctattcgaagtacactgcggatggaactgatggggtgcgatctgaacagttgttcaatgcccctgggaatggagtccaaggcaatctctgacgcccagattaccgctagctcctacttcactaatatgtttgctacctggagcccctccaaagcacgactgcatctgcagggacgaagcaacgcatggcgaccacaggtgaacaatcccaaggagtggctgcaggtcgattttcagaaaactatgaaggtgaccggagtcacaactcagggcgtgaaaagtctgctgacctcaatgtacgtcaaggagttcctgatctctagttcacaggacggccaccagtggacactgttctttcagaacggaaaggtgaaagtcttccagggcaatcaggattcctttacacctgtggtcaactctctggacccacccctgctgactcgctacctgcgaatccacccacagtcctgggtgcatcagattgcactgagaatggaagtcctgggctgcgaggcccaggacctgtattga

SEQ ID NO: 8 - DNA, 222 bp, Adeno-associated virus
gtctgtctgcacatttcgtagagcgagtgttccgatactctaatctccctaggcaaggttcatattgacttaggttacttattctccttttgttgactaagtcaataatcagaatcagcaggtttggagtcagcttggcagggatcagcagcctgggttggaaggagggggtataaaagccccttcaccaggagaagccgtcacacagatccacaagctcct

SEQ ID NO: 9 - DNA, 4778 bp, Adeno-associated virus
gtctgtctgcacatttcgtagagcgagtgttccgatactctaatctccctaggcaaggttcatattgacttaggttacttattctccttttgttgactaagtcaataatcagaatcagcaggtttggagtcagcttggcagggatcagcagcctgggttggaaggagggggtataaaagccccttcaccaggagaagccgtcacacagatccacaagctcctgctagcaggtaagtgccgtgtgtggttcccgcgggcctggcctctttacgggttatggcccttgcgtgccttgaattactgacactgacatccactttttctttttctccacaggtttaaacgccaccatgcagattgagctgtcaacttgctttttcctgtgcctgctgagattttgtttttccgctactagaagatactacctgggggctgtggaactgtcttgggattacatgcagagtgacctgggagagctgccagtggacgcacgatttccacctagagtccctaaatcattccccttcaacaccagcgtggtctataagaaaacactgttcgtggagtttactgatcacctgttcaacatcgctaagcctcggccaccctggatgggactgctgggaccaacaatccaggcagaggtgtacgacaccgtggtcattacactgaaaaacatggcctcacaccccgtgagcctgcatgctgtgggcgtcagctactggaaggcttccgaaggggcagagtatgacgatcagacttcccagagagaaaaagaggacgataaggtgtttcctggcgggtctcatacctatgtgtggcaggtcctgaaagagaatggccccatggcttccgaccctctgtgcctgacctactcttatctgagtcacgtggacctggtcaaggatctgaacagcggactgatcggagcactgctggtgtgtagggaagggagcctggctaaggagaaaacccagacactgcataagttcattctgctgttcgccgtgtttgacgaaggaaaatcatggcacagcgagacaaagaatagtctgatgcaggaccgggatgccgcttcagccagagcttggcccaaaatgcacactgtgaacggctacgtcaatcgctcactgcctggactgatcggctgccaccgaaagagcgtgtattggcatgtcatcggaatgggcaccacacctgaagtgcactccattttcctggaggggcatacctttctggtccgcaaccaccgacaggcctccctggagatctctccaattaccttcctgacagctcagactctgctgatggatctgggacagttcctgctgttttgccacatcagctcccaccagcatgatggcatggaggcctacgtgaaagtggacagctgtcccgaggaacctcagctgaggatgaagaacaatgaggaagctgaagactatgacgatgacctgaccgactccgagatggatgtggtccgattcgatgacgataacagcccctcctttatccagattagatctgtggccaagaaacaccctaagacatgggtccattacatcgcagccgaggaagaggactgggattatgcaccactggtgctggcaccagacgatcgatcctacaaatctcagtatctgaacaatggaccacagcggattggcagaaagtacaagaaagtgaggttcatggcttataccgatgaaaccttcaagactcgcgaagcaatccagcacgagagcgggattctgggaccactgctgtacggagaagtgggggacaccctgctgatcatttttaagaaccaggccagcaggccttacaatatctatccacatggaattacagatgtgcgccctctgtacagccggagactgccaaagggcgtcaaacacctgaaggacttcccaatcctgcccggggaaatttttaagtataaatggactgtcaccgtcgaggatggccccactaagagcgaccctaggtgcctgacccgctactattctagtttcgtgaatatggaaagggatctggccagcggactgatcggcccactgctgatttgttacaaagagagcgtggatcagagaggcaaccagatcatgtccgacaagaggaatgtgattctgttcagtgtctttgacgaaaaccggtcatggtatctgaccgagaacatccagagattcctgcctaatccagccggagtgcagctggaagatcctgagtttcaggcttctaacatcatgcatagtattaatggctacgtgttcgacagtctgcagctgtcagtgtgtctgcacgaggtcgcttactggtatatcctgagcattggagcacagacagatttcctgagcgtgttcttttccggctacacttttaagcataaaatggtgtatgaggacacactgactctgttccccttcagcggcgaaaccgtgtttatgtccatggagaatcccgggctgtggatcctgggatgccacaacagcgatttcaggaatcgcgggatgactgccctgctgaaagtgtcaagctgtgacaagaacaccggagactactatgaagattcatacgaggacatcagcgcatatctgctgtccaaaaacaatgccattgaacccaggtcttttagtcagaatcctccagtgctgaagaggcaccagcgcgagatcacccgcactaccctgcagagtgatcaggaagagatcgactacgacgatacaatttctgtggaaatgaagaaagaggacttcgatatctatgacgaagatgagaaccagagtcctcgatcattccagaagaaaacccggcattactttattgctgcagtggagcgcctgtgggattatggcatgtcctctagtcctcacgtgctgcgaaatcgggcccagtcagggagcgtcccacagttcaagaaagtggtcttccaggagtttacagacggatcctttactcagccactgtaccggggcgaactgaacgagcacctggggctgctgggaccctatatcagagctgaagtggaggataacattatggtcaccttcagaaatcaggcatctaggccttacagtttttattcaagcctgatctcttacgaagaggaccagaggcagggagcagaaccacgaaaaaacttcgtgaagcctaatgagaccaaaacatacttttggaaggtgcagcaccatatggccccaacaaaagacgaattcgattgcaaggcatgggcctatttttctgacgtggatctggagaaggacgtccacagtggcctgatcgggccactgctggtgtgtcatactaacaccctgaatcccgcacacggcaggcaggtcactgtccaggaattcgccctgttctttaccatctttgatgagacaaaaagctggtacttcaccgaaaacatggagcgaaattgccgggctccatgtaatattcagatggaagaccccacattcaaggagaactaccgctttcatgccatcaatgggtatattatggatactctgcccggactggtcatggctcaggaccagagaatcaggtggtacctgctgagcatggggtccaacgagaatatccactcaattcatttcagcggacacgtgtttactgtccggaagaaagaagagtataaaatggccctgtacaacctgtatcccggcgtgttcgaaaccgtcgagatgctgcctagcaaggcagggatctggagagtggaatgcctgattggggagcacctgcatgccggaatgtctaccctgtttctggtgtacagtaataagtgtcagacacccctggggatggcttccggacatatccgggatttccagattaccgcatctggacagtacggccagtgggcccctaagctggctagactgcactattccgggtctatcaacgcttggtccacaaaagagcctttctcttggattaaggtggacctgctggcaccaatgatcattcatggcatcaaaactcagggggccaggcagaagttctcctctctgtacatctcacagtttatcatcatgtacagcctggatggcaagaaatggcagacataccgcggcaatagcacagggactctgatggtgttctttggcaacgtggacagttcagggatcaagcacaacattttcaatccccctatcattgctagatacatcaggctgcacccaacccattattctattcgaagtacactgcggatggaactgatggggtgcgatctgaacagttgttcaatgcccctgggaatggagtccaaggcaatctctgacgcccagattaccgctagctcctacttcactaatatgtttgctacctggagcccctccaaagcacgactgcatctgcagggacgaagcaacgcatggcgaccacaggtgaacaatcccaaggagtggctgcaggtcgattttcagaaaactatgaaggtgaccggagtcacaactcagggcgtgaaaagtctgctgacctcaatgtacgtcaaggagttcctgatctctagttcacaggacggccaccagtggacactgttctttcagaacggaaaggtgaaagtcttccagggcaatcaggattcctttacacctgtggtcaactctctggacccacccctgctgactcgctacctgcgaatccacccacagtcctgggtgcatcagattgcactgagaatggaagtcctgggctgcgaggcccaggacctgtattgagcggccgcaataaaagatcagagctctagagatctgtgtgttggttttttgtgt

SEQ ID NO: 10 - DNA, 4374 bp, Adeno-associated virus
atgcagatcgagctgtctacctgcttcttcctgtgcctgctgcggttctgcttcagcgccaccagacggtactatctgggcgccgtggaactgagctgggactacatgcagagcgacctgggcgagctgcccgtggatgccagattccctccaagagtgcccaagagcttccccttcaacacctccgtggtgtacaagaaaaccctgttcgtggaattcaccgaccacctgttcaatatcgccaagcccagacccccctggatgggcctgctgggacctacaattcaggccgaggtgtacgacaccgtcgtgatcaccctgaagaacatggccagccaccccgtgtctctgcatgccgtgggagtgtcctactggaaggcctctgagggcgccgagtacgacgatcagaccagccagcgcgagaaagaggacgacaaggtgttccctggcggcagccacacctacgtgtggcaggtgctgaaagaaaacggccccatggcctccgaccctctgtgcctgacatacagctacctgagccacgtggacctcgtgaaggacctgaacagcggcctgatcggagccctgctcgtgtgtagagagggcagcctggccaaagagaaaacccagaccctgcacaagttcatcctgctgttcgccgtgttcgacgagggcaagagctggcacagcgagacaaagaacagcctgatgcaggaccgggacgccgcctctgctagagcctggcccaaaatgcacaccgtgaacggctacgtgaacagaagcctgcccggactgatcggctgccaccggaagtctgtgtactggcacgtgatcggcatgggcaccacccctgaggtgcacagcatctttctggaaggacacacctttctcgtgcggaaccaccggcaggccagcctggaaatcagccctatcaccttcctgaccgcccagacactgctgatggacctgggccagtttctgctgttctgccacatcagctcccaccagcacgacggcatggaagcctacgtgaaggtggacagctgccccgaggaaccccagctgcggatgaagaacaacgaggaagccgaggactacgacgacgacctgaccgacagcgagatggacgtggtgcgcttcgacgacgataacagccccagcttcatccagatcagaagcgtggccaagaagcaccccaagacctgggtgcactatatcgccgccgaggaagaggactgggattacgcccctctggtgctggcccccgacgacagaagctacaagagccagtacctgaacaatggcccccagcggatcggccggaagtataagaaagtgcggttcatggcctacaccgacgagacattcaagaccagagaggccatccagcacgagagcggcatcctgggccctctgctgtatggcgaagtgggcgacaccctgctgatcatcttcaagaaccaggccagcagaccctacaacatctaccctcacggcatcaccgacgtgcggcccctgtactctagaaggctgcccaagggcgtgaaacacctgaaggacttccccatcctgcccggcgagatcttcaagtacaagtggaccgtgaccgtggaagatggccccaccaagagcgaccccagatgcctgacacggtactacagcagcttcgtgaacatggaacgggacctggcctccggcctgattggcccactgctgatctgctacaaagaaagcgtggaccagcggggcaaccagatcatgagcgacaagcggaacgtgatcctgtttagcgtgttcgatgagaaccggtcctggtatctgaccgagaatatccagcggttcctgcccaaccctgccggcgtgcagctggaagatcctgagttccaggcctccaacatcatgcactccatcaatggctatgtgttcgacagcctgcagctgagcgtgtgcctgcacgaggtggcctactggtacatcctgagcatcggggcccagaccgacttcctgtccgtgttcttctccggctacaccttcaagcacaagatggtgtacgaggataccctgaccctgttcccctttagcggcgaaaccgtgttcatgagcatggaaaaccccggcctgtggatcctgggctgccacaacagcgacttccggaacagaggcatgaccgccctgctgaaggtgtccagctgcgacaagaacaccggcgactactacgaggacagctatgaggacatcagcgcctacctgctgagcaagaacaatgccatcgagcccagaagcttcagccagaacccccccgtgctgaagcggcaccagagagagatcacccggaccaccctgcagtccgaccaggaagagatcgattacgacgacaccatcagcgtggaaatgaagaaagaagatttcgacatctacgacgaggacgagaaccagagcccccggtcctttcagaaaaagacccggcactacttcattgccgctgtggaacggctgtgggactacggcatgagcagcagccctcacgtgctgagaaacagggcccagagcggcagcgtgccccagttcaagaaagtggtgttccaggaattcacagacggcagcttcacccagcctctgtaccgcggcgagctgaatgagcacctgggactgctgggcccctatatcagagccgaagtggaagataacatcatggtcaccttccggaatcaggcctcccggccctacagcttctacagctccctgatcagctacgaagaggaccagagacagggcgctgagccccggaagaacttcgtgaagcccaacgagactaagacctacttttggaaggtgcagcaccacatggcccctacaaaggacgagttcgactgcaaggcctgggcctacttctccgatgtggacctggaaaaggacgtgcactctgggctgatcggccccctgctcgtgtgccacaccaacaccctgaatcccgcccacggcagacaagtgacagtgcaggaattcgccctgttcttcaccatcttcgacgaaacaaagagctggtacttcaccgaaaacatggaaagaaactgccgggctccctgcaacatccagatggaagatcccaccttcaaagagaactaccggttccacgccatcaacggctacatcatggacacactgcccggcctcgtgatggctcaggatcagcggatccggtggtatctgctgtccatgggctccaacgagaacatccacagcatccacttcagcggccacgtgttcaccgtgcggaaaaaagaagagtacaaaatggccctgtacaacctgtaccctggggtgttcgagacagtggaaatgctgcccagcaaggccggcatctggcgggtggaatgtctgatcggcgagcatctgcacgctgggatgagcacactgtttctggtgtacagcaacaagtgccagacacctctgggcatggcctctggccacatccgggactttcagatcacagccagcggccagtatggccagtgggccccaaaactggccagactgcactacagcggcagcatcaacgcctggtccaccaaagagcccttcagctggatcaaggtggacctgctggctcccatgatcatccacggaatcaagacccagggcgccagacagaagttcagcagcctgtacatcagccagttcatcatcatgtacagcctggacggcaagaagtggcagacctaccggggcaatagcaccggcaccctgatggtgttcttcggcaacgtggactccagcggcattaagcacaacatcttcaacccccccatcattgcccggtacatccggctgcaccccacccactacagcatccggtccaccctgagaatggaactgatgggctgcgacctgaactcctgcagcatgcccctggggatggaaagcaaggccatctccgacgcccagatcaccgcctccagctacttcaccaacatgttcgccacctggtccccatccaaggcccggctgcatctgcagggcagaagcaatgcttggaggccccaagtgaacaaccccaaagaatggctgcaggtggacttccagaaaaccatgaaagtgaccggcgtgaccacccagggcgtgaagtctctgctgacctctatgtacgtgaaagagttcctgatctccagcagccaggacggccaccagtggaccctgtttttccagaacggcaaagtgaaagtgtttcaggggaaccaggactccttcacccccgtcgtgaatagcctggaccctccactgctgaccagatacctgcggatccaccctcagagttgggtgcaccagattgctctgcggatggaagtgctgggatgcgaggcccaggacctgtactga

SEQ ID NO: 11 - DNA, 4374 bp, Adeno-associated virus
atgcagatcgagctgtctacctgcttcttcctgtgcctgctgcggttctgctttagcgctactagacgctactacctgggcgccgtggaactgagctgggactatatgcagtcagacctgggcgagctgcccgtggacgctagattcccacctagagtgcctaagagcttcccctttaacacctccgtggtctataagaaaaccctgttcgtcgagttcaccgatcacctgtttaatatcgctaagcctagacccccctggatgggcctgctgggccctactattcaggccgaggtctacgacaccgtcgtgatcaccctgaagaatatggctagtcaccccgtcagcctgcacgccgtgggcgtcagctactggaaggctagcgagggcgccgagtacgacgatcagactagtcagcgcgagaaagaggacgacaaagtctttcctggcggctctcacacctacgtgtggcaggtcctgaaagaaaacggccctatggctagcgaccccctgtgcctgacctatagctacctgagtcacgtggacctggtcaaggacctgaatagcggcctgatcggcgccctgctcgtgtgtagagagggctcactggctaaagagaaaactcagaccctgcacaagtttatcctgctgttcgccgtgttcgacgagggcaagagctggcactcagagactaagaatagcctgatgcaggatagggacgccgctagcgctagagcctggcctaagatgcacaccgtgaacggctacgtgaacagatcactgcccggactgatcggctgtcaccggaagtccgtctactggcacgtgatcggaatgggcactacccccgaggtgcactctatctttctggaaggccacaccttcctcgtcagaaatcaccggcaggctagcctcgagattagccctatcaccttcctgaccgctcagacactgctgatggacctgggccagttcctgctgttttgtcacattagctctcaccagcacgacgggatggaagcctacgtgaaagtggatagctgccccgaggaacctcagctgagaatgaagaacaacgaggaagccgaggattacgacgacgacctgaccgatagcgagatggacgtcgtcagattcgacgacgataactcacctagctttattcagattagatcagtggctaagaagcaccctaagacctgggtgcactatatcgccgccgaggaagaggactgggactacgcccctctggtgctggcccccgacgatagaagctataagtctcagtacctgaacaacggccctcagcggatcggccggaagtataagaaagtgcggtttatggcctacaccgacgaaaccttcaagactagagaggctattcagcacgagtcagggatcctgggccccctgctctacggcgaagtgggcgacaccctgctgattatctttaagaatcaggctagtaggccctataatatctacccccacggaatcaccgacgtgcggcccctctactctagacggctgcctaagggcgtgaagcacctgaaggacttccctattctgcccggcgagatctttaagtacaagtggaccgtgaccgtcgaggacggccctactaagtccgaccctcggtgcctgactaggtactactctagcttcgtgaatatggaacgggacctggctagcggactgattggccctctgctgatctgctacaaagaatcagtggatcagcggggcaatcagattatgagcgataagcggaacgtgatcctgtttagtgtgtttgacgagaataggtcctggtatctgaccgagaatatccagcggttcctgcctaaccctgccggcgtgcagctggaagatcccgagtttcaggctagcaatattatgcactctattaacggatacgtgttcgatagcctgcagctgagcgtgtgcctgcacgaggtggcctactggtatatcctgtctatcggcgctcagaccgacttcctgagcgtgttctttagcggctacacctttaagcacaagatggtctacgaggataccctgaccctgttcccctttagcggcgaaaccgtgtttatgtctatggaaaaccccggcctgtggatcctggggtgtcacaatagcgactttaggaatagaggaatgaccgccctgctgaaagtgtctagctgcgataagaacaccggcgactattacgaggactcttacgaggatattagcgcctacctgctgtctaagaacaacgctatcgagcctagaagcttcagtcagaacccccccgtgctgaagcggcaccagagagagatcactagaactaccctgcagagcgaccaggaagagatcgactacgacgacactattagcgtcgagatgaagaaagaggatttcgatatctacgacgaggacgagaaccagtcacctagatccttccagaagaaaactaggcactactttattgccgccgtcgagcggctgtgggactacggaatgagttctagccctcacgtgctgagaaatagggctcagtcaggctcagtgcctcagttcaagaaagtggtgttccaggaattcaccgacggcagcttcactcagcccctctataggggcgagctgaacgagcacctgggactgctgggaccttatattagagccgaagtcgaggacaatattatggtcacctttaggaaccaggcctctaggccctacagcttctactctagcctgatcagctacgaggaagatcagcggcagggggccgaacctagaaagaacttcgtgaagcctaacgagactaagacctacttctggaaggtgcagcaccacatggcccctactaaggacgagttcgactgtaaagcctgggcctactttagcgacgtggacctcgagaaggacgtgcactcagggctgatcggacctctgctcgtctgtcacactaacaccctgaaccccgctcacggccggcaggtcacagtgcaggaattcgccctgttcttcactatcttcgacgaaactaagagctggtacttcacagagaatatggaaagaaactgtagggccccctgtaatattcagatggaagatcctacctttaaagagaactataggtttcacgctattaacggctatattatggacaccctgcccggcctcgtgatggctcaggatcagcggattaggtggtatctgctgtctatgggctctaacgagaatattcactctattcactttagcggccacgtgttcaccgtccggaagaaagaagagtataagatggccctctataacctctaccccggcgtgttcgagacagtggaaatgctgcctagtaaagccggaatctggcgggtcgagtgtctgatcggcgagcacctccacgccggaatgagcaccctgtttctggtctactctaacaagtgtcagacccctctgggaatggctagcggccacattagagactttcagatcaccgctagcggacagtacggccagtgggcccctaagctggctagactgcactatagcggatctatcaacgcctggtctaccaaagagccctttagctggattaaggtggacctgctggcccctatgattattcacgggattaagactcagggcgctaggcagaagtttagtagcctctatattagtcagtttatcattatgtatagcctggacggcaagaagtggcagacctatagaggcaatagcaccggcaccctgatggtgttcttcggcaacgtggactctagcgggatcaagcacaatatctttaacccccctattatcgctagatatattaggctgcaccctactcactactctattaggtctaccctgaggatggaactgatgggctgcgatctgaatagctgctctatgcccctggggatggaatctaaggctattagcgacgctcagatcacagcctctagctacttcactaatatgttcgctacctggtcccctagcaaggcccggctgcacctccagggcagatctaacgcttggcggcctcaggtcaacaaccctaaagagtggctgcaggtcgactttcagaaaactatgaaggtcaccggcgtgaccactcagggcgtgaaatcactgctgacctctatgtacgtgaaagagttcctgattagctctagccaggacggccaccagtggaccctgttctttcagaacggcaaagtgaaagtgtttcagggcaatcaggatagcttcacccccgtggtcaatagcctggatcccccactgctgactagatacctgagaattcaccctcagtcttgggtgcaccagatcgccctgagaatggaagtcctgggctgtgaagctcaggacctctactaa